European Patent Specification EP 3 743 514 B1, published June 26, 2024. Title: LACCASE VARIANTS WITH IMPROVED PROPERTIES. Applicant: Metgen OY. The sequence listing filed with the application follows.

SEQUENCE LISTING (67 sequences)

SEQ ID NO: 1 - protein, 512 aa, Bacillus wakoensis [sequence omitted]

SEQ ID NO: 2 - protein, 512 aa, Bacillus wakoensis
MRRKLEKFVDSLPIMETLQPKTKGKNYYEVKIQEFKKKLHRDLPPTTLWGYNAQFPGPTIEANSNEPVEVKWINELPNKHFLPVDWSIMNKDLPEVRHVTHLHGGRTPWVSDGYPEAWYTKDYKEVGSFFKEEVYRYLNEQRAMMLWYHDHTMGITRLNNYAGLAGAYIIRDKHEKSLNLPEGEYEVPLIIQDRTFNEDGSLFYPTGPEDGGEDLPNPSIVPAFLGDTVLVNGKVWPYLEVEPRKYRFRILNASNTRSYQLHLDSNQEVYQIGSDGGLLEKPVQMNKIPIESSERIDVIIDFSQCDGDEIVLKNDLGPDADAEDETNEIMKFKVSKPLKEKDTSVIPKRLSTIRSLRNNKISTHRNLKLVGSTDDFGRPLLLLNNKKWADPTTEKPKVGDTEVWSFINTTDFAHPMHIHLIHFQVLDRQPFDLERYNHDGTIIYTGPPRAPEPNERGWKDTVSAPAGQITRVIGTFAPYTGNYVWHCHILEHEDHDMMRPMKVIDPKQRKDK

SEQ ID NO: 3 - protein, 512 aa, Bacillus wakoensis
MRRKLEKFVDSLPIMETLQPKTKGKNYYEVKIQEFKKKLHRDLPPTTLWGYNAQFPGPTIEANSNEPVEVKWINELPNKHFLPVDWSIMNKDLPEVRHVTHLHGGRTPWVSDGYPEAWYTKDYKEVGPFFKEEVYRYLNEQRAMMLWYHDHTMGITRLNNYAGLAGAYIIRDKHEKSLNLPEGEYEVPLIIQDRTFNEDGSLFYPTGPEDGGEDLPNPSIVPAFLGDTVLVNGKVWPYLEVEPRKYRFRILNGSNTRSYQLHLDSNQEVYQIGSDGGLLEKPVQMNKIPIESSERIDVIIDFSQCDGDEIVLKNDLGPDADAEDETNEIMKFKVSKPLKEKDTSVIPKRLSTIRSLRNNKISTHRNLKLVGSTDDFGRPLLLLNNKKWADPTTEKPKVGDTEVWSFINTTDFAHPMHIHLIHFQVLDRQPFDLERYNHDGTIIYTGPPRAPEPNERGWKDTVSAPAGQITRVIGTFAPYTGNYVWHCHILEHEDHDMMRPMKVIDPKQRKDK

SEQ ID NO: 4 - protein, 512 aa, Bacillus wakoensis
MRRKLEKFVDSLPIMETLQPKTKGKNYYEVKIQEFKKKLHRDLPPTTLWGYNAQFPGPTIEANSNEPVEVKWINELPNKHFLPVDWSIMNKDLPEVRHVTHLHGGRTPWVSDGYPEAWYTKDYKEVGSFFKEEVYRYLNEQRAMMLWYHDHTMGITRLNNYAGLAGAYIIRDKHEKSLNLPEGEYEVPLIIQDRTFNEDGSLFYPTGPEDGGEDLPNPSIVPAFLGDTVLVNGKVWPYLEVEPRKYRFRILNGSNTRSYQLHLDSNQEVYQIGSDGGLLEKPVQMNKIPIESSERIDVIIDFSQCDGDEIVLKNDLGPDADAEDETNEIMKFKVSKPLKEKDTSVIPKRLSTIRSLRNNKISTHRNLKLVGSTDDFGRPLLLLDNKKWADPTTEKPKVGDTEVWSFINTTDFAHPMHIHLIHFQVLDRQPFDLERYNHDGTIIYTGPPRAPEPNERGWKDTVSAPAGQITRVIGTFAPYTGNYVWHCHILEHEDHDMMRPMKVIDPKQRKDK

SEQ ID NO: 5 - protein, 512 aa, Bacillus wakoensis
MRRKLEKFVDSLPIMETLQPKTKGKNYYEVKIQEFKKKLHRDLPPTTLWGYNAQFPGPTIEANSNEPVEVKWINELPNKHFLPVDWSIMNKDLPEVRHVTHLHGGRTPWVSDGYPEAWYTKDYKEVGSFFKEEVYRYLNEQRAMMLWYHDHTMGITRLNNYAGLAGAYIIRDKHEKSLNLPEGEYEVPLIIQDRTFNEDGSLFYPTGPEDGGEDLPNPSIVPAFLGDTVLVNGKVWPYLEVEPRKYRFRILNGSNTRSYQLHLDSNQEVYQIGSDGGLLEKPVQMNKIPIESSERIDVIIDFSQCDGDEIVLKNDLGPDADAEDETNEIMKFKVSKPLKEKDTSVIPKRLSTIRSLRNNKISTIRNLKLVGSTDDFGRPLLLLNNKKWADPTTEKPKVGDTEVWSFINTTDFAHPMHIHLIHFQVLDRQPFDLERYNHDGTIIYTGPPRAPEPNERGWKDTVSAPAGQITRVIGTFAPYTGNYVWHCHILEHEDHDMMRPMKVIDPKQRKDK

SEQ ID NO: 6 - protein, 512 aa, Bacillus wakoensis
MRRKLEKFVDSLPIMETLQPKTKGKNYYEVKIQEFKKKLHRDLPPTTLWGYNAQFPGPTIEANSNEPVEVKWINELPNKHFLPVDWSIMNKDLPEVRHVTHLHGGRTPWVSDGYPEAWYTKDYKEVGSFFKEEVYRYLNEQRAMMLWYHDHTMGITRLNNYAGLAGAYIIRDKHEKSLNLPEGEYEVPLIIQDRTFNEDGSLFYPTGPEDGGEDLPNPSIVPAFLGDTVLVNGKVWPYLEVEPRKYRFRILNGSNTRSYQLHLDSNQEVYQIGSDGGLLEKPVQMNKIPIEPSERIDVIIDFSQCDGDEIVLKNDLGPDADAEDETNEIMKFKVSKPLKEKDTSVIPKRLSTIRSLRNNKISTHRNLKLVGSTDDFGRPLLLLNNKKWADPTTEKPKVGDTEVWSFINTTDFAHPMHIHLIHFQVLDRQPFDLERYNHDGTIIYTGPPRAPEPNERGWKDTVSAPAGQITRVIGTFAPYTGNYVWHCHILEHEDHDMMRPMKVIDPKQRKDK

SEQ ID NO: 7 - protein, 512 aa, Bacillus wakoensis
MRRKLEKFVDSLPIMETLQPKTKGKNYYEVKIQEFKKKLHRDLPPTTLWGYNAQFPGPTIEANSNEPVEVKWINELPNKHFLPVDWSIMNKDLPEVRHVTHLHGGRTPWVSDGYPEAWYTKDYKEVGSFFKEEVYRYLNEQRAMMLWYHDHTMGITRLNNYAGLAGAYIIRDKHEKSLNLPEGEYEVPLIIQDRTFNEDGSLFYPTGPEDGGEDLPNPSIVPAFLGDTVLVNGKVWPYLEVEPRKYRFRILNGSNTRSYQLHLDSNQEVYQIGSDGGLLEKPVQMNKIPIESSERIDVIIDFSQCDGDEIVLKNDLGPDADAEDETNEIMKFKVSKPLKEKDTSVIPKRLSTIRSLRNNKISTHRNLKLVGSTDDFGRPLLLLNNKKWADPTTEKPKVGDTEVWSFINTTDFAHPMHIHLIHFQVLDRQPFDLERYNHDGTIIYTGPPRPPEPNERGWKDTVSAPAGQITRVIGTFAPYTGNYVWHCHILEHEDHDMMRPMKVIDPKQRKDK

SEQ ID NO: 8 - protein, 512 aa, Bacillus wakoensis
MRRKLEKFVDSLPIMETLQPKTKGKNYYEVKITEFKKKLHRDLPPTTLWGYNAQFPGPTIEANSNEPVEVKWINELPNKHFLPVDWSIMNKDLPEVRHVTHLHGGRTPWVSDGYPEAWYTKDYKEVGSFFKEEVYRYLNEQRAMMLWYHDHTMGITRLNNYAGLAGAYIIRDKHEKSLNLPEGEYEVPLIIQDRTFNEDGSLFYPTGPEDGGEDLPNPSIVPAFLGDTVLVNGKVWPYLEVEPRKYRFRILNGSNTRSYQLHLDSNQEVYQIGSDGGLLEKPVQMNKIPIESSERIDVIIDFSQCDGDEIVLKNDLGPDADAEDETNEIMKFKVSKPLKEKDTSVIPKRLSTIRSLRNNKISTHRNLKLVGSTDDFGRPLLLLNNKKWADPTTEKPKVGDTEVWSFINTTDFAHPMHIHLIHFQVLDRQPFDLERYNHDGTIIYTGPPRAPEPNERGWKDTVSAPAGQITRVIGTFAPYTGNYVWHCHILEHEDHDMMRPMKVIDPKQRKDK

SEQ ID NO: 9 - protein, 512 aa, Bacillus wakoensis
MRRKLEKFVDSLPIMETLQPKTKGKNYYEVKIQEFKKKLHRDLPPTTLWGYNAQFPGPTIEANSNEPVEVKWINELPNKHFLPVDWSIMNKDLPEVRHVTHLHGGRTPWVSDGYPEAWYTKDYKEVGSFFKEEVYRYLNEQRAMMLWYHDHTMGITRLNNYAGLAGAYIIRDKHEKSLNLPEGEYEVPLIIQDRTFNEDGSLFYPTGPEDGGEDLPNPSIVPAFLGDTVLVNGKVWPYLEVEPRKYRFRILNGSNTRSYQLHLDSNQEVYQIGSDGGLLEKPVQMNKIPIESSERIDVIIDFSQCDGDEIVLKNDLGPDADPEDETNEIMKFKVSKPLKEKDTSVIPKRLSTIRSLRNNKISTHRNLKLVGSTDDFGRPLLLLNNKKWADPTTEKPKVGDTEVWSFINTTDFAHPMHIHLIHFQVLDRQPFDLERYNHDGTIIYTGPPRAPEPNERGWKDTVSAPAGQITRVIGTFAPYTGNYVWHCHILEHEDHDMMRPMKVIDPKQRKDK

SEQ ID NO: 10 - protein, 512 aa, Bacillus wakoensis
MRRKLEKFVDSLPIMETLQPKTKGKNYYEVKIQEFKKKLHRDLPPTTLWGYNAQFPGPTIEANSNEPVEVKWINELPNKHFLPVDWSIMNKDLPEVRHVTHLHGGRTPWVSDGYPEAWYTKDYKEVGPFFKEEVYRYLNEQRAMMLWYHDHTMGITRLNNYAGLAGAYIIRDKHEKSLNLPEGEYEVPLIIQDRTFNEDGSLFYPTGPEDGGEDLPNPSIVPAFLGDTVLVNGKVWPYLEVEPRKYRFRILNASNTRSYQLHLDSNQEVYQIGSDGGLLEKPVQMNKIPIESSERIDVIIDFSQCDGDEIVLKNDLGPDADAEDETNEIMKFKVSKPLKEKDTSVIPKRLSTIRSLRNNKISTHRNLKLVGSTDDFGRPLLLLNNKKWADPTTEKPKVGDTEVWSFINTTDFAHPMHIHLIHFQVLDRQPFDLERYNHDGTIIYTGPPRAPEPNERGWKDTVSAPAGQITRVIGTFAPYTGNYVWHCHILEHEDHDMMRPMKVIDPKQRKDK

SEQ ID NO: 11 - protein, 512 aa, Bacillus wakoensis
MRRKLEKFVDSLPIMETLQPKTKGKNYYEVKIQEFKKKLHRDLPPTTLWGYNAQFPGPTIEANSNEPVEVKWINELPNKHFLPVDWSIMNKDLPEVRHVTHLHGGRTPWVSDGYPEAWYTKDYKEVGSFFKEEVYRYLNEQRAMMLWYHDHTMGITRLNNYAGLAGAYIIRDKHEKSLNLPEGEYEVPLIIQDRTFNEDGSLFYPTGPEDGGEDLPNPSIVPAFLGDTVLVNGKVWPYLEVEPRKYRFRILNASNTRSYQLHLDSNQEVYQIGSDGGLLEKPVQMNKIPIESSERIDVIIDFSQCDGDEIVLKNDLGPDADAEDETNEIMKFKVSKPLKEKDTSVIPKRLSTIRSLRNNKISTHRNLKLVGSTDDFGRPLLLLDNKKWADPTTEKPKVGDTEVWSFINTTDFAHPMHIHLIHFQVLDRQPFDLERYNHDGTIIYTGPPRAPEPNERGWKDTVSAPAGQITRVIGTFAPYTGNYVWHCHILEHEDHDMMRPMKVIDPKQRKDK

SEQ ID NO: 12 - protein, 512 aa, Bacillus wakoensis
MRRKLEKFVDSLPIMETLQPKTKGKNYYEVKIQEFKKKLHRDLPPTTLWGYNAQFPGPTIEANSNEPVEVKWINELPNKHFLPVDWSIMNKDLPEVRHVTHLHGGRTPWVSDGYPEAWYTKDYKEVGSFFKEEVYRYLNEQRAMMLWYHDHTMGITRLNNYAGLAGAYIIRDKHEKSLNLPEGEYEVPLIIQDRTFNEDGSLFYPTGPEDGGEDLPNPSIVPAFLGDTVLVNGKVWPYLEVEPRKYRFRILNASNTRSYQLHLDSNQEVYQIGSDGGLLEKPVQMNKIPIESSERIDVIIDFSQCDGDEIVLKNDLGPDADAEDETNEIMKFKVSKPLKEKDTSVIPKRLSTIRSLRNNKISTIRNLKLVGSTDDFGRPLLLLNNKKWADPTTEKPKVGDTEVWSFINTTDFAHPMHIHLIHFQVLDRQPFDLERYNHDGTIIYTGPPRAPEPNERGWKDTVSAPAGQITRVIGTFAPYTGNYVWHCHILEHEDHDMMRPMKVIDPKQRKDK

SEQ ID NO: 13 - protein, 512 aa, Bacillus wakoensis
MRRKLEKFVDSLPIMETLQPKTKGKNYYEVKIQEFKKKLHRDLPPTTLWGYNAQFPGPTIEANSNEPVEVKWINELPNKHFLPVDWSIMNKDLPEVRHVTHLHGGRTPWVSDGYPEAWYTKDYKEVGSFFKEEVYRYLNEQRAMMLWYHDHTMGITRLNNYAGLAGAYIIRDKHEKSLNLPEGEYEVPLIIQDRTFNEDGSLFYPTGPEDGGEDLPNPSIVPAFLGDTVLVNGKVWPYLEVEPRKYRFRILNASNTRSYQLHLDSNQEVYQIGSDGGLLEKPVQMNKIPIEPSERIDVIIDFSQCDGDEIVLKNDLGPDADAEDETNEIMKFKVSKPLKEKDTSVIPKRLSTIRSLRNNKISTHRNLKLVGSTDDFGRPLLLLNNKKWADPTTEKPKVGDTEVWSFINTTDFAHPMHIHLIHFQVLDRQPFDLERYNHDGTIIYTGPPRAPEPNERGWKDTVSAPAGQITRVIGTFAPYTGNYVWHCHILEHEDHDMMRPMKVIDPKQRKDK

SEQ ID NO: 14 - protein, 512 aa, Bacillus wakoensis
MRRKLEKFVDSLPIMETLQPKTKGKNYYEVKIQEFKKKLHRDLPPTTLWGYNAQFPGPTIEANSNEPVEVKWINELPNKHFLPVDWSIMNKDLPEVRHVTHLHGGRTPWVSDGYPEAWYTKDYKEVGSFFKEEVYRYLNEQRAMMLWYHDHTMGITRLNNYAGLAGAYIIRDKHEKSLNLPEGEYEVPLIIQDRTFNEDGSLFYPTGPEDGGEDLPNPSIVPAFLGDTVLVNGKVWPYLEVEPRKYRFRILNASNTRSYQLHLDSNQEVYQIGSDGGLLEKPVQMNKIPIESSERIDVIIDFSQCDGDEIVLKNDLGPDADAEDETNEIMKFKVSKPLKEKDTSVIPKRLSTIRSLRNNKISTHRNLKLVGSTDDFGRPLLLLNNKKWADPTTEKPKVGDTEVWSFINTTDFAHPMHIHLIHFQVLDRQPFDLERYNHDGTIIYTGPPRPPEPNERGWKDTVSAPAGQITRVIGTFAPYTGNYVWHCHILEHEDHDMMRPMKVIDPKQRKDK

SEQ ID NO: 15 - protein, 512 aa, Bacillus wakoensis
MRRKLEKFVDSLPIMETLQPKTKGKNYYEVKITEFKKKLHRDLPPTTLWGYNAQFPGPTIEANSNEPVEVKWINELPNKHFLPVDWSIMNKDLPEVRHVTHLHGGRTPWVSDGYPEAWYTKDYKEVGSFFKEEVYRYLNEQRAMMLWYHDHTMGITRLNNYAGLAGAYIIRDKHEKSLNLPEGEYEVPLIIQDRTFNEDGSLFYPTGPEDGGEDLPNPSIVPAFLGDTVLVNGKVWPYLEVEPRKYRFRILNASNTRSYQLHLDSNQEVYQIGSDGGLLEKPVQMNKIPIESSERIDVIIDFSQCDGDEIVLKNDLGPDADAEDETNEIMKFKVSKPLKEKDTSVIPKRLSTIRSLRNNKISTHRNLKLVGSTDDFGRPLLLLNNKKWADPTTEKPKVGDTEVWSFINTTDFAHPMHIHLIHFQVLDRQPFDLERYNHDGTIIYTGPPRAPEPNERGWKDTVSAPAGQITRVIGTFAPYTGNYVWHCHILEHEDHDMMRPMKVIDPKQRKDK

SEQ ID NO: 16 - protein, 512 aa, Bacillus wakoensis [sequence omitted]

SEQ ID NO: 17 - protein, 512 aa, Bacillus wakoensis
MRRKLEKFVDSLPIMETLQPKTKGKNYYEVKIQEFKKKLHRDLPPTTLWGYNAQFPGPTIEANSNEPVEVKWINELPNKHFLPVDWSIMNKDLPEVRHVTHLHGGRTPWVSDGYPEAWYTKDYKEVGPFFKEEVYRYLNEQRAMMLWYHDHTMGITRLNNYAGLAGAYIIRDKHEKSLNLPEGEYEVPLIIQDRTFNEDGSLFYPTGPEDGGEDLPNPSIVPAFLGDTVLVNGKVWPYLEVEPRKYRFRILNGSNTRSYQLHLDSNQEVYQIGSDGGLLEKPVQMNKIPIESSERIDVIIDFSQCDGDEIVLKNDLGPDADAEDETNEIMKFKVSKPLKEKDTSVIPKRLSTIRSLRNNKISTHRNLKLVGSTDDFGRPLLLLDNKKWADPTTEKPKVGDTEVWSFINTTDFAHPMHIHLIHFQVLDRQPFDLERYNHDGTIIYTGPPRAPEPNERGWKDTVSAPAGQITRVIGTFAPYTGNYVWHCHILEHEDHDMMRPMKVIDPKQRKDK

SEQ ID NO: 18 - protein, 512 aa, Bacillus wakoensis [sequence omitted]

SEQ ID NO: 19 - protein, 512 aa, Bacillus wakoensis
MRRKLEKFVDSLPIMETLQPKTKGKNYYEVKIQEFKKKLHRDLPPTTLWGYNAQFPGPTIEANSNEPVEVKWINELPNKHFLPVDWSIMNKDLPEVRHVTHLHGGRTPWVSDGYPEAWYTKDYKEVGPFFKEEVYRYLNEQRAMMLWYHDHTMGITRLNNYAGLAGAYIIRDKHEKSLNLPEGEYEVPLIIQDRTFNEDGSLFYPTGPEDGGEDLPNPSIVPAFLGDTVLVNGKVWPYLEVEPRKYRFRILNGSNTRSYQLHLDSNQEVYQIGSDGGLLEKPVQMNKIPIEPSERIDVIIDFSQCDGDEIVLKNDLGPDADAEDETNEIMKFKVSKPLKEKDTSVIPKRLSTIRSLRNNKISTHRNLKLVGSTDDFGRPLLLLNNKKWADPTTEKPKVGDTEVWSFINTTDFAHPMHIHLIHFQVLDRQPFDLERYNHDGTIIYTGPPRAPEPNERGWKDTVSAPAGQITRVIGTFAPYTGNYVWHCHILEHEDHDMMRPMKVIDPKQRKDK

SEQ ID NO: 20 - protein, 512 aa, Bacillus wakoensis
MRRKLEKFVDSLPIMETLQPKTKGKNYYEVKIQEFKKKLHRDLPPTTLWGYNAQFPGPTIEANSNEPVEVKWINELPNKHFLPVDWSIMNKDLPEVRHVTHLHGGRTPWVSDGYPEAWYTKDYKEVGPFFKEEVYRYLNEQRAMMLWYHDHTMGITRLNNYAGLAGAYIIRDKHEKSLNLPEGEYEVPLIIQDRTFNEDGSLFYPTGPEDGGEDLPNPSIVPAFLGDTVLVNGKVWPYLEVEPRKYRFRILNGSNTRSYQLHLDSNQEVYQIGSDGGLLEKPVQMNKIPIESSERIDVIIDFSQCDGDEIVLKNDLGPDADAEDETNEIMKFKVSKPLKEKDTSVIPKRLSTIRSLRNNKISTHRNLKLVGSTDDFGRPLLLLNNKKWADPTTEKPKVGDTEVWSFINTTDFAHPMHIHLIHFQVLDRQPFDLERYNHDGTIIYTGPPRPPEPNERGWKDTVSAPAGQITRVIGTFAPYTGNYVWHCHILEHEDHDMMRPMKVIDPKQRKDK

SEQ ID NO: 21 - protein, 512 aa, Bacillus wakoensis [sequence omitted]

SEQ ID NO: 22 - protein, 512 aa, Bacillus wakoensis [sequence omitted]

SEQ ID NO: 23 - protein, 512 aa, Bacillus wakoensis [sequence omitted]

SEQ ID NO: 24 - protein, 512 aa, Bacillus wakoensis
MRRKLEKFVDSLPIMETLQPKTKGKNYYEVKIQEFKKKLHRDLPPTTLWGYNAQFPGPTIEANSNEPVEVKWINELPNKHFLPVDWSIMNKDLPEVRHVTHLHGGRTPWVSDGYPEAWYTKDYKEVGSFFKEEVYRYLNEQRAMMLWYHDHTMGITRLNNYAGLAGAYIIRDKHEKSLNLPEGEYEVPLIIQDRTFNEDGSLFYPTGPEDGGEDLPNPSIVPAFLGDTVLVNGKVWPYLEVEPRKYRFRILNGSNTRSYQLHLDSNQEVYQIGSDGGLLEKPVQMNKIPIEPSERIDVIIDFSQCDGDEIVLKNDLGPDADAEDETNEIMKFKVSKPLKEKDTSVIPKRLSTIRSLRNNKISTHRNLKLVGSTDDFGRPLLLLDNKKWADPTTEKPKVGDTEVWSFINTTDFAHPMHIHLIHFQVLDRQPFDLERYNHDGTIIYTGPPRAPEPNERGWKDTVSAPAGQITRVIGTFAPYTGNYVWHCHILEHEDHDMMRPMKVIDPKQRKDK

SEQ ID NO: 25 - protein, 512 aa, Bacillus wakoensis [sequence omitted]

SEQ ID NO: 26 - protein, 512 aa, Bacillus wakoensis
MRRKLEKFVDSLPIMETLQPKTKGKNYYEVKITEFKKKLHRDLPPTTLWGYNAQFPGPTIEANSNEPVEVKWINELPNKHFLPVDWSIMNKDLPEVRHVTHLHGGRTPWVSDGYPEAWYTKDYKEVGSFFKEEVYRYLNEQRAMMLWYHDHTMGITRLNNYAGLAGAYIIRDKHEKSLNLPEGEYEVPLIIQDRTFNEDGSLFYPTGPEDGGEDLPNPSIVPAFLGDTVLVNGKVWPYLEVEPRKYRFRILNGSNTRSYQLHLDSNQEVYQIGSDGGLLEKPVQMNKIPIESSERIDVIIDFSQCDGDEIVLKNDLGPDADAEDETNEIMKFKVSKPLKEKDTSVIPKRLSTIRSLRNNKISTHRNLKLVGSTDDFGRPLLLLDNKKWADPTTEKPKVGDTEVWSFINTTDFAHPMHIHLIHFQVLDRQPFDLERYNHDGTIIYTGPPRAPEPNERGWKDTVSAPAGQITRVIGTFAPYTGNYVWHCHILEHEDHDMMRPMKVIDPKQRKDK

SEQ ID NO: 27 - protein, 512 aa, Bacillus wakoensis
MRRKLEKFVDSLPIMETLQPKTKGKNYYEVKIQEFKKKLHRDLPPTTLWGYNAQFPGPTIEANSNEPVEVKWINELPNKHFLPVDWSIMNKDLPEVRHVTHLHGGRTPWVSDGYPEAWYTKDYKEVGSFFKEEVYRYLNEQRAMMLWYHDHTMGITRLNNYAGLAGAYIIRDKHEKSLNLPEGEYEVPLIIQDRTFNEDGSLFYPTGPEDGGEDLPNPSIVPAFLGDTVLVNGKVWPYLEVEPRKYRFRILNGSNTRSYQLHLDSNQEVYQIGSDGGLLEKPVQMNKIPIESSERIDVIIDFSQCDGDEIVLKNDLGPDADPEDETNEIMKFKVSKPLKEKDTSVIPKRLSTIRSLRNNKISTHRNLKLVGSTDDFGRPLLLLDNKKWADPTTEKPKVGDTEVWSFINTTDFAHPMHIHLIHFQVLDRQPFDLERYNHDGTIIYTGPPRAPEPNERGWKDTVSAPAGQITRVIGTFAPYTGNYVWHCHILEHEDHDMMRPMKVIDPKQRKDK

SEQ ID NO: 28 - protein, 512 aa, Bacillus wakoensis [sequence omitted]

SEQ ID NO: 29 - protein, 512 aa, Bacillus wakoensis
MRRKLEKFVDSLPIMETLQPKTKGKNYYEVKIQEFKKKLHRDLPPTTLWGYNAQFPGPTIEANSNEPVEVKWINELPNKHFLPVDWSIMNKDLPEVRHVTHLHGGRTPWVSDGYPEAWYTKDYKEVGSFFKEEVYRYLNEQRAMMLWYHDHTMGITRLNNYAGLAGAYIIRDKHEKSLNLPEGEYEVPLIIQDRTFNEDGSLFYPTGPEDGGEDLPNPSIVPAFLGDTVLVNGKVWPYLEVEPRKYRFRILNGSNTRSYQLHLDSNQEVYQIGSDGGLLEKPVQMNKIPIESSERIDVIIDFSQCDGDEIVLKNDLGPDADAEDETNEIMKFKVSKPLKEKDTSVIPKRLSTIRSLRNNKISTIRNLKLVGSTDDFGRPLLLLNNKKWADPTTEKPKVGDTEVWSFINTTDFAHPMHIHLIHFQVLDRQPFDLERYNHDGTIIYTGPPRPPEPNERGWKDTVSAPAGQITRVIGTFAPYTGNYVWHCHILEHEDHDMMRPMKVIDPKQRKDK

SEQ ID NO: 30 - protein, 512 aa, Bacillus wakoensis
MRRKLEKFVDSLPIMETLQPKTKGKNYYEVKITEFKKKLHRDLPPTTLWGYNAQFPGPTIEANSNEPVEVKWINELPNKHFLPVDWSIMNKDLPEVRHVTHLHGGRTPWVSDGYPEAWYTKDYKEVGSFFKEEVYRYLNEQRAMMLWYHDHTMGITRLNNYAGLAGAYIIRDKHEKSLNLPEGEYEVPLIIQDRTFNEDGSLFYPTGPEDGGEDLPNPSIVPAFLGDTVLVNGKVWPYLEVEPRKYRFRILNGSNTRSYQLHLDSNQEVYQIGSDGGLLEKPVQMNKIPIESSERIDVIIDFSQCDGDEIVLKNDLGPDADAEDETNEIMKFKVSKPLKEKDTSVIPKRLSTIRSLRNNKISTIRNLKLVGSTDDFGRPLLLLNNKKWADPTTEKPKVGDTEVWSFINTTDFAHPMHIHLIHFQVLDRQPFDLERYNHDGTIIYTGPPRAPEPNERGWKDTVSAPAGQITRVIGTFAPYTGNYVWHCHILEHEDHDMMRPMKVIDPKQRKDK

SEQ ID NO: 31 - protein, 512 aa, Bacillus wakoensis
MRRKLEKFVDSLPIMETLQPKTKGKNYYEVKIQEFKKKLHRDLPPTTLWGYNAQFPGPTIEANSNEPVEVKWINELPNKHFLPVDWSIMNKDLPEVRHVTHLHGGRTPWVSDGYPEAWYTKDYKEVGSFFKEEVYRYLNEQRAMMLWYHDHTMGITRLNNYAGLAGAYIIRDKHEKSLNLPEGEYEVPLIIQDRTFNEDGSLFYPTGPEDGGEDLPNPSIVPAFLGDTVLVNGKVWPYLEVEPRKYRFRILNGSNTRSYQLHLDSNQEVYQIGSDGGLLEKPVQMNKIPIESSERIDVIIDFSQCDGDEIVLKNDLGPDADPEDETNEIMKFKVSKPLKEKDTSVIPKRLSTIRSLRNNKISTIRNLKLVGSTDDFGRPLLLLNNKKWADPTTEKPKVGDTEVWSFINTTDFAHPMHIHLIHFQVLDRQPFDLERYNHDGTIIYTGPPRAPEPNERGWKDTVSAPAGQITRVIGTFAPYTGNYVWHCHILEHEDHDMMRPMKVIDPKQRKDK

SEQ ID NO: 32 - protein, 512 aa, Bacillus wakoensis [sequence omitted]

SEQ ID NO: 33 - protein, 512 aa, Bacillus wakoensis [sequence omitted]

SEQ ID NO: 34 - protein, 512 aa, Bacillus wakoensis
MRRKLEKFVDSLPIMETLQPKTKGKNYYEVKIQEFKKKLHRDLPPTTLWGYNAQFPGPTIEANSNEPVEVKWINELPNKHFLPVDWSIMNKDLPEVRHVTHLHGGRTPWVSDGYPEAWYTKDYKEVGSFFKEEVYRYLNEQRAMMLWYHDHTMGITRLNNYAGLAGAYIIRDKHEKSLNLPEGEYEVPLIIQDRTFNEDGSLFYPTGPEDGGEDLPNPSIVPAFLGDTVLVNGKVWPYLEVEPRKYRFRILNGSNTRSYQLHLDSNQEVYQIGSDGGLLEKPVQMNKIPIEPSERIDVIIDFSQCDGDEIVLKNDLGPDADPEDETNEIMKFKVSKPLKEKDTSVIPKRLSTIRSLRNNKISTHRNLKLVGSTDDFGRPLLLLNNKKWADPTTEKPKVGDTEVWSFINTTDFAHPMHIHLIHFQVLDRQPFDLERYNHDGTIIYTGPPRAPEPNERGWKDTVSAPAGQITRVIGTFAPYTGNYVWHCHILEHEDHDMMRPMKVIDPKQRKDK

SEQ ID NO: 35 - protein, 512 aa, Bacillus wakoensis
MRRKLEKFVDSLPIMETLQPKTKGKNYYEVKITEFKKKLHRDLPPTTLWGYNAQFPGPTIEANSNEPVEVKWINELPNKHFLPVDWSIMNKDLPEVRHVTHLHGGRTPWVSDGYPEAWYTKDYKEVGSFFKEEVYRYLNEQRAMMLWYHDHTMGITRLNNYAGLAGAYIIRDKHEKSLNLPEGEYEVPLIIQDRTFNEDGSLFYPTGPEDGGEDLPNPSIVPAFLGDTVLVNGKVWPYLEVEPRKYRFRILNGSNTRSYQLHLDSNQEVYQIGSDGGLLEKPVQMNKIPIESSERIDVIIDFSQCDGDEIVLKNDLGPDADAEDETNEIMKFKVSKPLKEKDTSVIPKRLSTIRSLRNNKISTHRNLKLVGSTDDFGRPLLLLNNKKWADPTTEKPKVGDTEVWSFINTTDFAHPMHIHLIHFQVLDRQPFDLERYNHDGTIIYTGPPRPPEPNERGWKDTVSAPAGQITRVIGTFAPYTGNYVWHCHILEHEDHDMMRPMKVIDPKQRKDK

SEQ ID NO: 36 - protein, 512 aa, Bacillus wakoensis
MRRKLEKFVDSLPIMETLQPKTKGKNYYEVKIQEFKKKLHRDLPPTTLWGYNAQFPGPTIEANSNEPVEVKWINELPNKHFLPVDWSIMNKDLPEVRHVTHLHGGRTPWVSDGYPEAWYTKDYKEVGSFFKEEVYRYLNEQRAMMLWYHDHTMGITRLNNYAGLAGAYIIRDKHEKSLNLPEGEYEVPLIIQDRTFNEDGSLFYPTGPEDGGEDLPNPSIVPAFLGDTVLVNGKVWPYLEVEPRKYRFRILNGSNTRSYQLHLDSNQEVYQIGSDGGLLEKPVQMNKIPIESSERIDVIIDFSQCDGDEIVLKNDLGPDADPEDETNEIMKFKVSKPLKEKDTSVIPKRLSTIRSLRNNKISTHRNLKLVGSTDDFGRPLLLLNNKKWADPTTEKPKVGDTEVWSFINTTDFAHPMHIHLIHFQVLDRQPFDLERYNHDGTIIYTGPPRPPEPNERGWKDTVSAPAGQITRVIGTFAPYTGNYVWHCHILEHEDHDMMRPMKVIDPKQRKDK

SEQ ID NO: 37 - protein, 512 aa, Bacillus wakoensis [sequence omitted]

SEQ ID NO: 38 - protein, 512 aa, Bacillus wakoensis
MRRKLEKFVDSLPIMETLQPKTKGKNYYEVKIQEFKKKLHRDLPPTTLWGYNAQFPGPTIEANSNEPVEVKWINELPNKHFLPVDWSIMNKDLPEVRHVTHLHGGRTPWVSDGYPEAWYTKDYKEVGPFFKEEVYRYLNEQRAMMLWYHDHTMGITRLNNYAGLAGAYIIRDKHEKSLNLPEGEYEVPLIIQDRTFNEDGSLFYPTGPEDGGEDLPNPSIVPAFLGDTVLVNGKVWPYLEVEPRKYRFRILNASNTRSYQLHLDSNQEVYQIGSDGGLLEKPVQMNKIPIESSERIDVIIDFSQCDGDEIVLKNDLGPDADAEDETNEIMKFKVSKPLKEKDTSVIPKRLSTIRSLRNNKISTHRNLKLVGSTDDFGRPLLLLDNKKWADPTTEKPKVGDTEVWSFINTTDFAHPMHIHLIHFQVLDRQPFDLERYNHDGTIIYTGPPRAPEPNERGWKDTVSAPAGQITRVIGTFAPYTGNYVWHCHILEHEDHDMMRPMKVIDPKQRKDK

SEQ ID NO: 39 - protein, 512 aa, Bacillus wakoensis
MRRKLEKFVDSLPIMETLQPKTKGKNYYEVKIQEFKKKLHRDLPPTTLWGYNAQFPGPTIEANSNEPVEVKWINELPNKHFLPVDWSIMNKDLPEVRHVTHLHGGRTPWVSDGYPEAWYTKDYKEVGPFFKEEVYRYLNEQRAMMLWYHDHTMGITRLNNYAGLAGAYIIRDKHEKSLNLPEGEYEVPLIIQDRTFNEDGSLFYPTGPEDGGEDLPNPSIVPAFLGDTVLVNGKVWPYLEVEPRKYRFRILNASNTRSYQLHLDSNQEVYQIGSDGGLLEKPVQMNKIPIESSERIDVIIDFSQCDGDEIVLKNDLGPDADAEDETNEIMKFKVSKPLKEKDTSVIPKRLSTIRSLRNNKISTIRNLKLVGSTDDFGRPLLLLDNKKWADPTTEKPKVGDTEVWSFINTTDFAHPMHIHLIHFQVLDRQPFDLERYNHDGTIIYTGPPRAPEPNERGWKDTVSAPAGQITRVIGTFAPYTGNYVWHCHILEHEDHDMMRPMKVIDPKQRKDK

SEQ ID NO: 40 - protein, 512 aa, Bacillus wakoensis
MRRKLEKFVDSLPIMETLQPKTKGKNYYEVKIQEFKKKLHRDLPPTTLWGYNAQFPGPTIEANSNEPVEVKWINELPNKHFLPVDWSIMNKDLPEVRHVTHLHGGRTPWVSDGYPEAWYTKDYKEVGPFFKEEVYRYLNEQRAMMLWYHDHTMGITRLNNYAGLAGAYIIRDKHEKSLNLPEGEYEVPLIIQDRTFNEDGSLFYPTGPEDGGEDLPNPSIVPAFLGDTVLVNGKVWPYLEVEPRKYRFRILNASNTRSYQLHLDSNQEVYQIGSDGGLLEKPVQMNKIPIEPSERIDVIIDFSQCDGDEIVLKNDLGPDADAEDETNEIMKFKVSKPLKEKDTSVIPKRLSTIRSLRNNKISTIRNLKLVGSTDDFGRPLLLLDNKKWADPTTEKPKVGDTEVWSFINTTDFAHPMHIHLIHFQVLDRQPFDLERYNHDGTIIYTGPPRAPEPNERGWKDTVSAPAGQITRVIGTFAPYTGNYVWHCHILEHEDHDMMRPMKVIDPKQRKDK

SEQ ID NO: 41 - protein, 512 aa, Bacillus wakoensis [sequence omitted]

SEQ ID NO: 42 - protein, 512 aa, Bacillus wakoensis
MRRKLEKFVDSLPIMETLQPKTKGKNYYEVKITEFKKKLHRDLPPTTLWGYNAQFPGPTIEANSNEPVEVKWINELPNKHFLPVDWSIMNKDLPEVRHVTHLHGGRTPWVSDGYPEAWYTKDYKEVGPFFKEEVYRYLNEQRAMMLWYHDHTMGITRLNNYAGLAGAYIIRDKHEKSLNLPEGEYEVPLIIQDRTFNEDGSLFYPTGPEDGGEDLPNPSIVPAFLGDTVLVNGKVWPYLEVEPRKYRFRILNASNTRSYQLHLDSNQEVYQIGSDGGLLEKPVQMNKIPIEPSERIDVIIDFSQCDGDEIVLKNDLGPDADAEDETNEIMKFKVSKPLKEKDTSVIPKRLSTIRSLRNNKISTIRNLKLVGSTDDFGRPLLLLDNKKWADPTTEKPKVGDTEVWSFINTTDFAHPMHIHLIHFQVLDRQPFDLERYNHDGTIIYTGPPRPPEPNERGWKDTVSAPAGQITRVIGTFAPYTGNYVWHCHILEHEDHDMMRPMKVIDPKQRKDK

SEQ ID NO: 43 - protein, 512 aa, Bacillus wakoensis
MRRKLEKFVDSLPIMETLQPKTKGKNYYEVKITEFKKKLHRDLPPTTLWGYNAQFPGPTIEANSNEPVEVKWINELPNKHFLPVDWSIMNKDLPEVRHVTHLHGGRTPWVSDGYPEAWYTKDYKEVGPFFKEEVYRYLNEQRAMMLWYHDHTMGITRLNNYAGLAGAYIIRDKHEKSLNLPEGEYEVPLIIQDRTFNEDGSLFYPTGPEDGGEDLPNPSIVPAFLGDTVLVNGKVWPYLEVEPRKYRFRILNASNTRSYQLHLDSNQEVYQIGSDGGLLEKPVQMNKIPIEPSERIDVIIDFSQCDGDEIVLKNDLGPDADPEDETNEIMKFKVSKPLKEKDTSVIPKRLSTIRSLRNNKISTIRNLKLVGSTDDFGRPLLLLDNKKWADPTTEKPKVGDTEVWSFINTTDFAHPMHIHLIHFQVLDRQPFDLERYNHDGTIIYTGPPRPPEPNERGWKDTVSAPAGQITRVIGTFAPYTGNYVWHCHILEHEDHDMMRPMKVIDPKQRKDK

SEQ ID NO: 44 - protein, 507 aa, Bacillus salsus
MSPKLEKFVDQLPILAALKPNRREADGDYYEITMEEFFQKLHRDLPPTRLWGYNRQVPGPTLDVIQDEPIKVKWVNNLPSRHFLPVDKSFLMPDLPEVRTVTHLHGGETPPPSDGYPEAWFTRNYAEVGPFFEREVYEYLNQQRATMLWYHDHAMGTTRLNNYAGLAGAYIIRDKYEKSLNLPSGEYEIPLIIQDKSFNRDGSLSYPKQPDNASEDLPNPSVVPAFFGDTILVNGKVWPFLKVEPRKYRFRMLNASNTRGYQLHLDSEQPFYQIGSDGGLLEKPVKLNMITIEPSERMDIILDFSKYEGKDIILRNNLGPNADPENETDEVMKFIVSKPLKEQDKSVIPKRLSTIPSLRANQISAYRNLKLVGSQDEYGRPLLLLNNKRWADPITEKPRLGTTEIWSFINTTAFAHPMHIHLIQFQVLERQPFDLDRYNEDGQIIFTGAPKPPEPNERGWKDTIKATSGHITRVIGKYGPFTGNYVWHCHILEHEDHDMMRPFKVIE

SEQ ID NO: 45 - DNA, 24 bp, artificial sequence
  primer
gaaattaatacgactcactatagg

SEQ ID NO: 46 - DNA, 27 bp, artificial sequence
  primer
ggttatgctagttattgctcagcggtg

SEQ ID NO: 47 - DNA, 30 bp, Bacillus spec
attcagaatacgaaaacgatatttacgcgg

SEQ ID NO: 48 - DNA, 35 bp, Bacillus spec
atcgttttcgtattctgaatgctagcaacacccgt

SEQ ID NO: 49 - DNA, 30 bp, Bacillus spec
gcccacttctttataatctttcgtatacca

SEQ ID NO: 50 - DNA, 35 bp, Bacillus spec
aagattataaagaagtgggccccttcttcaaagaa

SEQ ID NO: 51 - DNA, 30 bp, Bacillus spec
cagcagcagcagaggacgaccaaaatcatc

SEQ ID NO: 52 - DNA, 35 bp, Bacillus spec
gtcgtcctctgctgctgctggacaacaaaaaatgg

SEQ ID NO: 53 - DNA, 30 bp, Bacillus spec
ggtgctaattttgttattacgcaggctacg

SEQ ID NO: 54 - DNA, 35 bp, Bacillus spec
gtaataacaaaattagcaccattcgtaatctgaaa

SEQ ID NO: 55 - DNA, 30 bp, Bacillus spec
ttcaatcggaattttgttcatctgcaccgg

SEQ ID NO: 56 - DNA, 35 bp, Bacillus spec
tgaacaaaattccgattgaacccagcgaacgcatt

SEQ ID NO: 57 - DNA, 30 bp, Bacillus spec
acgaggcggaccggtatagataatggtgcc

SEQ ID NO: 58 - DNA, 35 bp, Bacillus spec
tctataccggtccgcctcgtccaccggaaccgaat

SEQ ID NO: 59 - DNA, 30 bp, Bacillus spec
gattttcacctcataatagtttttgccttt

SEQ ID NO: 60 - DNA, 35 bp, Bacillus spec
actattatgaggtgaaaatcacagagtttaaaaaa

SEQ ID NO: 61 - DNA, 30 bp, Bacillus spec
atctgcatccggacccagatcatttttcag

SEQ ID NO: 62 - DNA, 35 bp, Bacillus spec
atctgggtccggatgcagatcccgaagatgaaacc

SEQ ID NO: 63 - protein, 13 aa, artificial sequence
  primer
MRRKLEKFVDSLP

SEQ ID NO: 64 - protein, 11 aa, artificial sequence
  primer
MRRKKFVDSLP

SEQ ID NO: 65 - protein, 509 aa, Bacillus clausii
MELEKFVDPMPIMKTAIPKKTSKDGDYYEIEMKEFSQKLHRDLNPTRLWGYDGQFPGPTIEVMRGKPARIKWMNNLPDTHFLPIDRSIHHVAHEPEVRTVVHLHGSETTPASDGYPEAWFTKDFAEVGSFFEQETYEYPNDQRAATLWYHDHAMGITRLNVYAGLSGLYIIRDPREEQLNLPKGEFDIPLLIQDRSFNDDGSLFYPAQPANPAPNLPNPSVLPFFVGDTILVNGKVWPYLQVEPRKYRFRILNGSNSRSYQLALDSEAPFYQIASDGGLLRRTVSLQAFDIRPAERIEAIIDFSKFEGQTITLKNNASTDATADVMQFQVVLPLSGEDTSIIPQNLSYIPSLQQNDVKRIRNLKISGTTDEYGRPLLLLNNKLWSDPVEEKPCLGTTEIWSFVNVTNVPHPMHIHLVQFQLLDHRAFNVELYNENGQIELVGPTIPPKINERGWKDTITAPAGQITRVIARFAPFSGYYVWHCHILEHEDYDMMRPFVVIDPKTEKERR

SEQ ID NO: 66 - protein, 513 aa, Bacillus subtilis
MTLEKFVDALPIPDTLKPVQQTTEKTYYEVTMEECAHQLHRDLPPTRLWGYNGLFPGPTIEVKRNENVYVKWMNNLPSEHFLPIDHTIHHSDSQHEEPEVKTVVHLHGGVTPPDSDGYPEAWFSKDFEQTGPYFKREVYHYPNQQRGATLWYHDHAMALTRLNVYAGLVGAYIIHDPKEKRLKLPSGEYDVPLLITDRTINEDGSLFYPSGPENPSPSLPKPSIVPAFCGDTILVNGKVWPYLEVEPRKYRFRVINASNARTYNLSLDNGGEFIQIGSDGGLLPRSVKLNSFSLAPAERYDIIIDFTAYEGESIILANSEGCGGDANPETDANIMQFRVTKPLAQKDESRKPKYLASYPSVQNERIQNIRTLKLAGTQDEYGRVVQLLNNKRWHDPVTEAPKAGTTEIWSIVNPTQGTHPIHLHLVSFRVLDRRPFDIARYQERGELSYTGPAVPPPPSEKGWKDTIQAHAGEVLRIAVTFGPYSGRYVWHCHILEHEDYDMMRPMDITDPHK

SEQ ID NO: 67 - protein, 519 aa, Escherichia coli
MQRRDFLKYSVALGVASALPLWNRAVFAAERPTLPIPDLLTTDARNRIQLTIGAGQSTFGGKTATTWGYNGNLLGPAVKLQRGKAVTVDIYNQLTEETTLHWHGLEVPGEVDGGPQGIIPPGGKRSVTLNVDQPAATCWFHPHQHGKTGRQVAMGLAGLVVIEDDEILKLMLPKQWGIDDVPVIVQDKKFSADGQIDYQLDVMTAAVGWFGDTLLTNGAIYPQHAAPRGWLRLRLLNGCNARSLNFATSDNRPLYVIASDGGLLPEPVKVSELPVLMGERFEVLVEVNDNKPFDLVTLPVSQMGMAIAPFDKPHPVMRIQPIAISASGALPDTLSSLPALPSLEGLTVRKLQLSMDPMLDMMGMQMLMEKYGDQAMAGMDHSQMMGHMGHGNMNHMNHGGKFDFHHANKINGQAFDMNKPMFAAAKGQYERWVISGVGDMMLHPFHIHGTQFRILSENGKPPAAHRAGWKDTVKVEGNVSEVLVKFNHDAPKEHAYMAHCHLLEHEDTGMMLGFTVSDP